European Patent Specification EP 3 458 116 B1, published March 13, 2024. Title: SPIDER SILK COATING OF SOLID SURFACES. Applicant: Spiber Technologies AB. The sequence listing filed with the application follows.

SEQUENCE LISTING (72 sequences)

SEQ ID NO: 1 - DNA, 789 bp, Euprosthenops australis
ggtccgaattcaggtcaaggaggatatggtggactaggtcaaggagggtatggacaaggtgcaggaagttctgcagccgctgccgccgccgcagcagccgccgcagcaggtggacaaggtggacaaggtcaaggaggatatggacaaggttcaggaggttctgcagccgccgccgccgccgcagcagcagcagcagctgcagcagctggacgaggtcaaggaggatatggccaaggttctggaggtaatgctgctgccgcagccgctgccgccgccgccgccgctgcagcagccggacagggaggtcaaggtggatatggtagacaaagccaaggtgctggttccgctgctgctgctgctgctgctgctgccgctgctgctgctgcaggatctggacaaggtggatacggtggacaaggtcaaggaggttatggtcagagtagtgcttctgcttcagctgctgcgtcagctgctagtactgtagctaattcggtgagtcgcctctcatcgccttccgcagtatctcgagtttcttcagcagtttctagcttggtttcaaatggtcaagtgaatatggcagcgttacctaatatcatttccaacatttcttcttctgtcagtgcatctgctcctggtgcttctggatgtgaggtcatagtgcaagctctactcgaagtcatcactgctcttgttcaaatcgttagttcttctagtgttggatatattaatccatctgctgtgaaccaaattactaatgttgttgctaatgccatggctcaagtaatgggc

SEQ ID NO: 2 - protein, 263 aa, Euprosthenops australis
  DOMAIN (1)..(158): REP fragment
  DOMAIN (159)..(165): Spacer fragment
  DOMAIN (166)..(263): CT fragment
GPNSGQGGYGGLGQGGYGQGAGSSAAAAAAAAAAAAGGQGGQGQGGYGQGSGGSAAAAAAAAAAAAAAAGRGQGGYGQGSGGNAAAAAAAAAAAAAAAGQGGQGGYGRQSQGAGSAAAAAAAAAAAAAAGSGQGGYGGQGQGGYGQSSASASAAASAASTVANSVSRLSSPSAVSRVSSAVSSLVSNGQVNMAALPNIISNISSSVSASAPGASGCEVIVQALLEVITALVQIVSSSSVGYINPSAVNQITNVVANAMAQVMG

SEQ ID NO: 3 - protein, 98 aa, Euprosthenops australis
SRLSSPSAVSRVSSAVSSLVSNGQVNMAALPNIISNISSSVSASAPGASGCEVIVQALLEVITALVQIVSSSSVGYINPSAVNQITNVVANAMAQVMG

SEQ ID NO: 4 - protein, 100 aa, Artificial Sequence
  Consensus sequence derived from known MaSp1 and MaSp2 proteins
  MISC_FEATURE (1)..(71): Sequence length present in known species variants
  VARIANT (7)..(7): Glu
SRLSSPQASSRVSSAVSNLVSSGPTNSAALSNTISNVVSQISASNPGLSGCDVLVQALLEVVSALVHILGSSSIGQVNYGSAGQATQIVGQSVAQALGEF

SEQ ID NO: 5 - protein, 1110 aa, Euprosthenops australis
  REPEAT (7)..(19)
  REPEAT (20)..(42)
  REPEAT (43)..(56)
  REPEAT (57)..(70)
  REPEAT (71)..(83)
  REPEAT (84)..(106)
  REPEAT (107)..(120)
  REPEAT (121)..(134)
  REPEAT (135)..(147)
  REPEAT (148)..(170)
  REPEAT (171)..(183)
  REPEAT (184)..(197)
  REPEAT (198)..(211)
  REPEAT (212)..(234)
  REPEAT (235)..(248)
  REPEAT (249)..(265)
  REPEAT (266)..(279)
  REPEAT (280)..(293)
  REPEAT (294)..(306)
  REPEAT (307)..(329)
  REPEAT (330)..(342)
  REPEAT (343)..(356)
  REPEAT (357)..(370)
  REPEAT (371)..(393)
  REPEAT (394)..(406)
  REPEAT (407)..(420)
  REPEAT (421)..(434)
  REPEAT (435)..(457)
  REPEAT (458)..(470)
  REPEAT (471)..(488)
  REPEAT (489)..(502)
  REPEAT (503)..(516)
  REPEAT (517)..(529)
  REPEAT (530)..(552)
  REPEAT (553)..(566)
  REPEAT (567)..(580)
  REPEAT (581)..(594)
  REPEAT (595)..(617)
  REPEAT (618)..(630)
  REPEAT (631)..(647)
  REPEAT (648)..(661)
  REPEAT (662)..(675)
  REPEAT (676)..(688)
  REPEAT (689)..(711)
  REPEAT (712)..(725)
  REPEAT (726)..(739)
  REPEAT (740)..(752)
  REPEAT (753)..(775)
  REPEAT (776)..(789)
  REPEAT (790)..(803)
  REPEAT (804)..(816)
  REPEAT (817)..(839)
  REPEAT (840)..(853)
  REPEAT (854)..(867)
  REPEAT (868)..(880)
  REPEAT (881)..(903)
  REPEAT (904)..(917)
  REPEAT (918)..(931)
  REPEAT (932)..(945)
  REPEAT (946)..(968)
  REPEAT (969)..(981)
  REPEAT (982)..(998)
  REPEAT (999)..(1013)
  REPEAT (1014)..(1027)
  REPEAT (1028)..(1042)
  REPEAT (1043)..(1059)
  REPEAT (1060)..(1073)
  REPEAT (1074)..(1092)
QGAGGNAAAAAAAAAAAAAGQGGQGGYGGLGQGGYGQGAGSSAAAAAAAAAAAAAAGRGQGGYGQGSGGNAAAAAAAAAAAASGQGGQGGQGGQGQGGYGQGAGSSAAAAAAAAAAAAAAGQGQGRYGQGAGGNAAAAAAAAAAAAAGQGGQGGQGGLGQGGYGQGAGSSAAAAAASAAAAAAGRGQGGYGQGAGGNAAAAAAAAAAAAAAGQGGQGGYGGLGQGGYGQGAGSSAAAAAAAAAAAAAGGQGGQGQGRYGQGAGSSAAAAAAAAAAAAAAGQGQGGYGQGAGGNAAAAAAAAAAAAAGQGGQGGQGGLGQGGYGQGAGSSAAAAAAAAAAAAAGRGQGGYGQGAGGNAAAAAAAAAEAAAAGQGGQGGYGGLGQGGYGQGAGSSAAAAAAAAAAAAAGRGQGGYGQGAGGNAAAAAAAAAAAAAAGQGGQGGYGGLGQGGYGQGAGSSAAAAAAAAAAAAAGGQGGQGQGRYGQGAGSSAAAAAAAAAAAAAAGRGQGGYGQGSGGNAAAAAAAAAAAASGQGSQGGQGGQGQGGYGQGAGSSAAAAAAAAAAAAASGRGQGGYGQGAGGNAAAAAAAAAAAAAAGQGGQGGYGGLGQGGYGQGAGSSAAAAAAAAAAAAGGQGGQGQGGYGQGAGSSAAAAAAAAAAAAAAGRGQGGYGQGSGGNAAAAAAAAAAAASGQGGQGGQGGQGQGGYGQGAGSSAAAAAAAAAAAAAAGQGQGGYGQGAGGNAAAAAAAAAAAAAGQGGQGGQGGLGQGGYGQGAGSSAAAAAAAAAAAAAAGRGQGGYGQGVGGNAAAAAAAAAAAAAGQGGQGGQGGLGQGGYGQGAGSSAAAAAAAAAAAAAAGRGQGGYGQGSGGNAAAAAAAAAAAASGQGSQGGQGGQGQGGYGQGAGSSAAAAAAAAAAAAASGRGQGGYGQGAGGNAAAAAAAAAAAAAAGQGGQGGYGGLGQGGYGQGAGSSAAAAAAAAAAAAGGQGGQGQGGYGQGSGGSAAAAAAAAAAAAAAAGRGQGGYGQGSGGNAAAAAAAAAAAAAAAGQGGQGGYGRQSQGAGSAAAAAAAAAAAAAAGSGQGGYGGQGQGGYGQSSASASAAASAASTVANSVS

SEQ ID NO: 6 - protein, 23 aa, Artificial Sequence
  Consensus sequence derived from internal repeats of Euprosthenops australis MaSp1
  VARIANT (4)..(4): Ser
  VARIANT (8)..(8): Tyr
  VARIANT (11)..(11): Gln
GQGGQGGQGGLGQGGYGQGAGSS

SEQ ID NO: 7 - protein, 17 aa, Artificial Sequence
  Consensus sequence derived from internal repeats of Euprosthenops australis MaSp1
  VARIANT (9)..(9): Arg
  VARIANT (14)..(14): Ser
  VARIANT (16)..(16): Gly
GQGGQGQGGYGQGAGSS

SEQ ID NO: 8 - protein, 14 aa, Artificial Sequence
  Consensus sequence derived from internal repeats of Euprosthenops australis MaSp1
  VARIANT (2)..(2): Gln
  VARIANT (6)..(6): Arg
  VARIANT (11)..(11): Ser
  VARIANT (11)..(11): Val
GRGQGGYGQGAGGN

SEQ ID NO: 9 - protein, 290 aa, Artificial Sequence
  Fusion protein
GPNSGIGKFLHSAGKFGKAFVGEIMKSGSASGQGGYGGLGQGGYGQGAGSSAAAAAAAAAAAAGGQGGQGQGGYGQGSGGSAAAAAAAAAAAAAAAGRGQGGYGQGSGGNAAAAAAAAAAAAAAAGQGGQGGYGRQSQGAGSAAAAAAAAAAAAAAGSGQGGYGGQGQGGYGQSSASASAAASAASTVANSVSRLSSPSAVSRVSSAVSSLVSNGQVNMAALPNIISNISSSVSASAPGASGCEVIVQALLEVITALVQIVSSSSVGYINPSAVNQITNVVANAMAQVMG

SEQ ID NO: 10 - DNA, 870 bp, Artificial Sequence
  Fusion protein
ggtccgaattcaggaattggtaaatttttgcactcagcaggaaaatttggaaaagcttttgtgggagagataatgaaatcaggatccgctagcggtcaaggaggatatggtggactaggtcaaggagggtatggacaaggtgcaggaagttctgcagccgctgccgccgccgcagcagccgccgcagcaggtggacaaggtggacaaggtcaaggaggatatggacaaggttcaggaggttctgcagccgccgccgccgccgcagcagcagcagcagctgcagcagctggacgaggtcaaggaggatatggccaaggttctggaggtaatgctgctgccgcagccgctgccgccgccgccgccgctgcagcagccggacagggaggtcaaggtggatatggtagacaaagccaaggtgctggttccgctgctgctgctgctgctgctgctgccgctgctgctgctgcaggatctggacaaggtggatacggtggacaaggtcaaggaggttatggtcagagtagtgcttctgcttcagctgctgcgtcagctgctagtactgtagctaattcggtgagtcgcctctcatcgccttccgcagtatctcgagtttcttcagcagtttctagcttggtttcaaatggtcaagtgaatatggcagcgttacctaatatcatttccaacatttcttcttctgtcagtgcatctgctcctggtgcttctggatgtgaggtcatagtgcaagctctactcgaagtcatcactgctcttgttcaaatcgttagttcttctagtgttggatatattaatccatctgctgtgaaccaaattactaatgttgttgctaatgccatggctcaagtaatgggc

SEQ ID NO: 11 - protein, 277 aa, Artificial Sequence
  Fusion protein
  DISULFID (5)..(14)
GPNSCTGRGDSPACGSASGQGGYGGLGQGGYGQGAGSSAAAAAAAAAAAAGGQGGQGQGGYGQGSGGSAAAAAAAAAAAAAAAGRGQGGYGQGSGGNAAAAAAAAAAAAAAAGQGGQGGYGRQSQGAGSAAAAAAAAAAAAAAGSGQGGYGGQGQGGYGQSSASASAAASAASTVANSVSRLSSPSAVSRVSSAVSSLVSNGQVNMAALPNIISNISSSVSASAPGASGCEVIVQALLEVITALVQIVSSSSVGYINPSAVNQITNVVANAMAQVMG

SEQ ID NO: 12 - DNA, 831 bp, Artificial Sequence
  Fusion protein
ggtccgaattcatgcacaggtcgtggtgattctccggcgtgcggatccgctagcggtcaaggaggatatggtggactaggtcaaggagggtatggacaaggtgcaggaagttctgcagccgctgccgccgccgcagcagccgccgcagcaggtggacaaggtggacaaggtcaaggaggatatggacaaggttcaggaggttctgcagccgccgccgccgccgcagcagcagcagcagctgcagcagctggacgaggtcaaggaggatatggccaaggttctggaggtaatgctgctgccgcagccgctgccgccgccgccgccgctgcagcagccggacagggaggtcaaggtggatatggtagacaaagccaaggtgctggttccgctgctgctgctgctgctgctgctgccgctgctgctgctgcaggatctggacaaggtggatacggtggacaaggtcaaggaggttatggtcagagtagtgcttctgcttcagctgctgcgtcagctgctagtactgtagctaattcggtgagtcgcctctcatcgccttccgcagtatctcgagtttcttcagcagtttctagcttggtttcaaatggtcaagtgaatatggcagcgttacctaatatcatttccaacatttcttcttctgtcagtgcatctgctcctggtgcttctggatgtgaggtcatagtgcaagctctactcgaagtcatcactgctcttgttcaaatcgttagttcttctagtgttggatatattaatccatctgctgtgaaccaaattactaatgttgttgctaatgccatggctcaagtaatgggc

SEQ ID NO: 13 - protein, 339 aa, Artificial Sequence
  Fusion protein
MGSSGHHHHHHMVDNKFNKEQQNAFYEILHLPNLNEEQRNAFIQSLKDDPSQSANLLAEAKKLNDAQAPKLEALFQGPNSGQGGYGGLGQGGYGQGAGSSAAAAAAAAAAAAGGQGGQGQGGYGQGSGGSAAAAAAAAAAAAAAAGRGQGGYGQGSGGNAAAAAAAAAAAAAAAGQGGQGGYGRQSQGAGSAAAAAAAAAAAAAAGSGQGGYGGQGQGGYGQSSASASAAASAASTVANSVSRLSSPSAVSRVSSAVSSLVSNGQVNMAALPNIISNISSSVSASAPGASGCEVIVQALLEVITALVQIVSSSSVGYINPSAVNQITNVVANAMAQVMG

SEQ ID NO: 14 - DNA, 1017 bp, Artificial Sequence
  Fusion protein
atgggcagcagcggccatcatcatcatcatcatatggtagacaacaaattcaacaaagaacaacaaaacgcgttctatgagatcttacatttacctaacttaaacgaagaacaacgaaacgccttcatccaaagtttaaaagatgacccaagccaaagcgctaacttgctagcagaagctaaaaagctaaatgatgctcaggcgccgaaactggaagctctgttccagggtccgaattcaggtcaaggtggatatggtggactaggtcaaggaggatatggacaaggtgcaggaagttctgcagccgctgccgccgccgcagcagccgccgcagcaggtggacaaggtggacaaggtcaaggaggatatggacaaggttcaggaggttctgcagccgccgccgccgccgcagcagcagcagcagctgcagcagctggacgaggtcaaggaggatatggtcaaggttctggaggtaatgctgctgccgcagccgctgccgccgccgccgccgctgcagcagccggacagggaggtcaaggtggatatggtagacaaagccaaggtgctggttccgctgctgctgctgctgctgctgctgccgctgctgctgctgcaggatctggacaaggtggatacggtggacaaggtcaaggaggttatggtcagagtagtgcttctgcttcagctgctgcgtcagctgctagtactgtagctaattcggtgagtcgcctctcatcgccttccgcagtatctcgagtttcttcagcagtttctagcttggtttcaaatggtcaagtgaatatggcagcgttacctaatatcatttccaacatttcttcttctgtcagtgcatctgctcctggtgcttctggatgtgaggtcatagtgcaagctctactcgaagtcatcactgctcttgttcaaatcgttagttcttctagtgttggatatattaatccatctgctgtgaaccaaattactaatgttgttgctaatgccatggctcaagtaatgggc

SEQ ID NO: 15 - protein, 336 aa, Artificial Sequence
  Fusion protein
MGSSGHHHHHHMTYKLVINGKTLKGETTTEAVDAATAEKVFKQYANDNGVDGEWTYDDATKTFTVTELEALFQGPNSGQGGYGGLGQGGYGQGAGSSAAAAAAAAAAAAGGQGGQGQGGYGQGSGGSAAAAAAAAAAAAAAAGRGQGGYGQGSGGNAAAAAAAAAAAAAAAGQGGQGGYGRQSQGAGSAAAAAAAAAAAAAAGSGQGGYGGQGQGGYGQSSASASAAASAASTVANSVSRLSSPSAVSRVSSAVSSLVSNGQVNMAALPNIISNISSSVSASAPGASGCEVIVQALLEVITALVQIVSSSSVGYINPSAVNQITNVVANAMAQVMG

SEQ ID NO: 16 - DNA, 1008 bp, Artificial Sequence
  Fusion protein
atgggcagcagcggccatcatcatcatcatcatatgacttacaaacttgttattaatggtaaaacattgaaaggcgaaacaactactgaagctgttgatgctgctactgcagaaaaagtcttcaaacaatacgctaacgacaacggtgttgacggtgaatggacttacgacgatgcgactaagacctttacagttactgaactggaagctctgttccagggtccgaattcaggtcaaggtggatatggtggactaggtcaaggaggatatggacaaggtgcaggaagttctgcagccgctgccgccgccgcagcagccgccgcagcaggtggacaaggtggacaaggtcaaggaggatatggacaaggttcaggaggttctgcagccgccgccgccgccgcagcagcagcagcagctgcagcagctggacgaggtcaaggaggatatggtcaaggttctggaggtaatgctgctgccgcagccgctgccgccgccgccgccgctgcagcagccggacagggaggtcaaggtggatatggtagacaaagccaaggtgctggttccgctgctgctgctgctgctgctgctgccgctgctgctgctgcaggatctggacaaggtggatacggtggacaaggtcaaggaggttatggtcagagtagtgcttctgcttcagctgctgcgtcagctgctagtactgtagctaattcggtgagtcgcctctcatcgccttccgcagtatctcgagtttcttcagcagtttctagcttggtttcaaatggtcaagtgaatatggcagcgttacctaatatcatttccaacatttcttcttctgtcagtgcatctgctcctggtgcttctggatgtgaggtcatagtgcaagctctactcgaagtcatcactgctcttgttcaaatcgttagttcttctagtgttggatatattaatccatctgctgtgaaccaaattactaatgttgttgctaatgccatggctcaagtaatgggc

SEQ ID NO: 17 - protein, 327 aa, Artificial Sequence
  Fusion protein
MGSSGHHHHHHMLAEAKVLANRELDKYGVSDYYKNLINNAKTVEGVKALIDEILAALPLEALFQGPNSGQGGYGGLGQGGYGQGAGSSAAAAAAAAAAAAGGQGGQGQGGYGQGSGGSAAAAAAAAAAAAAAAGRGQGGYGQGSGGNAAAAAAAAAAAAAAAGQGGQGGYGRQSQGAGSAAAAAAAAAAAAAAGSGQGGYGGQGQGGYGQSSASASAAASAASTVANSVSRLSSPSAVSRVSSAVSSLVSNGQVNMAALPNIISNISSSVSASAPGASGCEVIVQALLEVITALVQIVSSSSVGYINPSAVNQITNVVANAMAQVMG

SEQ ID NO: 18 - DNA, 981 bp, Artificial Sequence
  Fusion protein
atgggcagcagcggccatcatcatcatcatcatatgttagctgaagctaaagtcttagctaacagagaacttgacaaatatggagtaagtgactattacaagaacctaatcaacaatgccaaaactgttgaaggtgtaaaagcactgatagatgaaattttagctgcattacctctggaagctctgttccagggtccgaattcaggtcaaggtggatatggtggactaggtcaaggaggatatggacaaggtgcaggaagttctgcagccgctgccgccgccgcagcagccgccgcagcaggtggacaaggtggacaaggtcaaggaggatatggacaaggttcaggaggttctgcagccgccgccgccgccgcagcagcagcagcagctgcagcagctggacgaggtcaaggaggatatggtcaaggttctggaggtaatgctgctgccgcagccgctgccgccgccgccgccgctgcagcagccggacagggaggtcaaggtggatatggtagacaaagccaaggtgctggttccgctgctgctgctgctgctgctgctgccgctgctgctgctgcaggatctggacaaggtggatacggtggacaaggtcaaggaggttatggtcagagtagtgcttctgcttcagctgctgcgtcagctgctagtactgtagctaattcggtgagtcgcctctcatcgccttccgcagtatctcgagtttcttcagcagtttctagcttggtttcaaatggtcaagtgaatatggcagcgttacctaatatcatttccaacatttcttcttctgtcagtgcatctgctcctggtgcttctggatgtgaggtcatagtgcaagctctactcgaagtcatcactgctcttgttcaaatcgttagttcttctagtgttggatatattaatccatctgctgtgaaccaaattactaatgttgttgctaatgccatggctcaagtaatgggc

SEQ ID NO: 19 - protein, 429 aa, Artificial Sequence
  Fusion protein
MHHHHHHGQGGYGGLGQGGYGQGAGSSAAAAAAAAAAAAGGQGGQGQGGYGQGSGGSAAAAAAAAAAAAAAAGRGQGGYGQGSGGNAAAAAAAAAAAAAAAGQGGQGGYGRQSQGAGSAAAAAAAAAAAAAAGSGQGGYGGQGQGGYGQSSASASAAASAASTVANSVSRLSSPSAVSRVSSAVSSLVSNGQVNMAALPNIISNISSSVSASAPGASGCEVIVQALLEVITALVQIVSSSSVGYINPSAVNQITNVVANAMAQVMGGNSGSGSGSAAGSITTLPALPEDGGSGAFPPGHFKDPKRLYCKNGGFFLRIHPDGRVDGVREKSDPHIKLQLQAEERGVVSIKGVCANRYLAMKEDGRLLASKCVTDECFFFERLESNNYNTYRSRKYTSWYVALKRTGQYKLGSKTGPGQKAILFLPMSAKS

SEQ ID NO: 20 - DNA, 1287 bp, Artificial Sequence
  Fusion protein
atgcatcatcatcatcatcatggtcaaggtggatatggtggactaggtcaaggaggatatggacaaggtgcaggaagttctgcagccgctgccgccgccgcagcagccgccgcagcaggtggacaaggtggacaaggtcaaggaggatatggacaaggttcaggaggttctgcagccgccgccgccgccgcagcagcagcagcagctgcagcagctggacgaggtcaaggaggatatggtcaaggttctggaggtaatgctgctgccgcagccgctgccgccgccgccgccgctgcagcagccggacagggaggtcaaggtggatatggtagacaaagccaaggtgctggttccgctgctgctgctgctgctgctgctgccgctgctgctgctgcaggatctggacaaggtggatacggtggacaaggtcaaggaggttatggtcagagtagtgcttctgcttcagctgctgcgtcagctgctagtactgtagctaattcggtgagtcgcctctcatcgccttccgcagtatctcgagtttcttcagcagtttctagcttggtttcaaatggtcaagtgaatatggcagcgttacctaatatcatttccaacatttcttcttctgtcagtgcatctgctcctggtgcttctggatgtgaggtcatagtgcaagctctactcgaagtcatcactgctcttgttcaaatcgttagttcttctagtgttggatatattaatccatctgctgtgaaccaaattactaatgttgttgctaatgccatggctcaagtaatgggcgggaattcaggtagcggcagcggtagcgcagccgggagcatcaccacgctgcccgccttgcccgaggatggcggcagcggcgccttcccgcccggccacttcaaggaccccaagcggctgtactgcaaaaacgggggcttcttcctgcgcatccaccccgacggccgagttgacggggtccgggagaagagcgaccctcacatcaagctacaacttcaagcagaagagagaggagttgtgtctatcaaaggagtgtgtgctaaccgttacctggctatgaaggaagatggaagattactggcttctaaatgtgttacggatgagtgtttcttttttgaacgattggaatctaataactacaatacttaccggtcaaggaaatacaccagttggtatgtggcactgaaacgaactgggcagtataaacttggatccaaaacaggacctgggcagaaagctatactttttcttccaatgtctgctaagagc

SEQ ID NO: 21 - protein, 427 aa, Artificial Sequence
  Fusion protein
MGSSGHHHHHHMMGKISSLPTQLFKCCFCDFLKVKMHTMSSSHLFYLALCLLTFTSSATAGPETLCGAELVDALQFVCGDRGFYFNKPTGYGSSSRRAPQTGIVDECCFRSCDLRRLEMYCAPLKPAKSARSVRAQRHTDMPKTQKEVHLKNASRGSAGNKNYRMPNSGQGGYGGLGQGGYGQGAGSSAAAAAAAAAAAAGGQGGQGQGGYGQGSGGSAAAAAAAAAAAAAAAGRGQGGYGQGSGGNAAAAAAAAAAAAAAAGQGGQGGYGRQSQGAGSAAAAAAAAAAAAAAGSGQGGYGGQGQGGYGQSSASASAAASAASTVANSVSRLSSPSAVSRVSSAVSSLVSNGQVNMAALPNIISNISSSVSASAPGASGCEVIVQALLEVITALVQIVSSSSVGYINPSAVNQITNVVANAMAQVMG

SEQ ID NO: 22 - DNA, 1281 bp, Artificial Sequence
  Fusion protein
atgggcagcagcggccatcatcatcatcatcatatgatgggaaaaatcagcagtcttccaacccaattatttaagtgctgcttttgtgatttcttgaaggtgaagatgcacaccatgtcctcctcgcatctcttctacctggcgctgtgcctgctcaccttcaccagctctgccacggctggaccggagacgctctgcggggctgagctggtggatgctcttcagttcgtgtgtggagacaggggcttttatttcaacaagcccacagggtatggctccagcagtcggagggcgcctcagacaggtatcgtggatgagtgctgcttccggagctgtgatctaaggaggctggagatgtattgcgcacccctcaagcctgccaagtcagctcgctctgtccgtgcccagcgccacaccgacatgcccaagacccagaaggaagtacatttgaagaacgcaagtagagggagtgcaggaaacaagaactacaggatgccgaattcaggtcaaggtggatatggtggactaggtcaaggaggatatggacaaggtgcaggaagttctgcagccgctgccgccgccgcagcagccgccgcagcaggtggacaaggtggacaaggtcaaggaggatatggacaaggttcaggaggttctgcagccgccgccgccgccgcagcagcagcagcagctgcagcagctggacgaggtcaaggaggatatggtcaaggttctggaggtaatgctgctgccgcagccgctgccgccgccgccgccgctgcagcagccggacagggaggtcaaggtggatatggtagacaaagccaaggtgctggttccgctgctgctgctgctgctgctgctgccgctgctgctgctgcaggatctggacaaggtggatacggtggacaaggtcaaggaggttatggtcagagtagtgcttctgcttcagctgctgcgtcagctgctagtactgtagctaattcggtgagtcgcctctcatcgccttccgcagtatctcgagtttcttcagcagtttctagcttggtttcaaatggtcaagtgaatatggcagcgttacctaatatcatttccaacatttcttcttctgtcagtgcatctgctcctggtgcttctggatgtgaggtcatagtgcaagctctactcgaagtcatcactgctcttgttcaaatcgttagttcttctagtgttggatatattaatccatctgctgtgaaccaaattactaatgttgttgctaatgccatggctcaagtaatgggc

SEQ ID NO: 23 - protein, 641 aa, Artificial Sequence
  Fusion protein
MGSSGHHHHHHMNCCVKGNSIYPQKTSTKQTGLMLDIARHFYSPEVIKSFIDTISLSGGNFLHLHFSDHENYAIESHLLNQRAENAVQGKDGIYINPYTGKPFLSYRQLDDIKAYAKAKGIELIPELDSPNHMTAIFKLVQKDRGVKYLQGLKSRQVDDEIDITNADSITFMQSLMSEVIDIFGDTSQHFHIGGDEFGYSVESNHEFITYANKLSYFLEKKGLKTRMWNDGLIKNTFEQINPNIEITYWSYDGDTQDKNEAAERRDMRVSLPELLAKGFTVLNYNSYYLYIVPKASPTFSQDAAFAAKDVIKNWDLGVWDGRNTKNRVQNTHEIAGAALSIWGEDAKALKDETIQKNTKSLLEAVIHKTNGDEGPAALGPNSGQGGYGGLGQGGYGQGAGSSAAAAAAAAAAAAGGQGGQGQGGYGQGSGGSAAAAAAAAAAAAAAAGRGQGGYGQGSGGNAAAAAAAAAAAAAAAGQGGQGGYGRQSQGAGSAAAAAAAAAAAAAAGSGQGGYGGQGQGGYGQSSASASAAASAASTVANSVSRLSSPSAVSRVSSAVSSLVSNGQVNMAALPNIISNISSSVSASAPGASGCEVIVQALLEVITALVQIVSSSSVGYINPSAVNQITNVVANAMAQVMG

SEQ ID NO: 24 - DNA, 1923 bp, Artificial Sequence
  Fusion protein
atgggcagcagcggccatcatcatcatcatcatatgaactgctgcgtgaaaggcaacagcatttatccgcagaaaaccagcaccaaacagaccggcctgatgctggatattgcgcgccatttttatagcccggaagtgattaaaagctttattgataccattagcctgagcggcggcaactttctgcatctgcattttagcgatcatgaaaactatgcgattgaaagccatctgctgaaccagcgcgcggaaaacgcggtgcagggcaaagatggcatttatattaacccgtataccggcaaaccgtttctgagctatcgccagctggatgatattaaagcgtatgcgaaagcgaaaggcattgaactgattccggaactggatagcccgaaccacatgaccgcgatttttaaactggtgcagaaagatcgcggcgtgaaatatctgcagggcctgaaaagccgccaggtggatgatgaaattgatattaccaacgcggatagcattacctttatgcagagcctgatgagcgaagtgattgatatttttggcgataccagccagcattttcatattggcggcgatgaatttggctatagcgtggaaagcaaccatgaatttattacctatgcgaacaaactgagctattttctggaaaaaaaaggcctgaaaacccgcatgtggaacgatggcctgattaaaaacacctttgaacagattaacccgaacattgaaattacctattggagctatgatggcgatacccaggataaaaacgaagcggcggaacgccgcgatatgcgcgtgagcctgccggaactgctggcgaaaggctttaccgtgctgaactataacagctattatctgtatattgtgccgaaagcgagcccgacctttagccaggatgcggcgtttgcggcgaaagatgtgattaaaaactgggatctgggcgtgtgggatggccgcaacaccaaaaaccgcgtgcagaacacccatgaaattgcgggcgcggcgctgagcatttggggcgaagatgcgaaagcgctgaaagatgaaaccattcagaaaaacaccaaaagcctgctggaagcggtgattcataaaaccaacggcgatgaaggcccggcggcgctgggcccgaattcaggtcaaggtggatatggtggactaggtcaaggaggatatggacaaggtgcaggaagttctgcagccgctgccgccgccgcagcagccgccgcagcaggtggacaaggtggacaaggtcaaggaggatatggacaaggttcaggaggttctgcagccgccgccgccgccgcagcagcagcagcagctgcagcagctggacgaggtcaaggaggatatggtcaaggttctggaggtaatgctgctgccgcagccgctgccgccgccgccgccgctgcagcagccggacagggaggtcaaggtggatatggtagacaaagccaaggtgctggttccgctgctgctgctgctgctgctgctgccgctgctgctgctgcaggatctggacaaggtggatacggtggacaaggtcaaggaggttatggtcagagtagtgcttctgcttcagctgctgcgtcagctgctagtactgtagctaattcggtgagtcgcctctcatcgccttccgcagtatctcgagtttcttcagcagtttctagcttggtttcaaatggtcaagtgaatatggcagcgttacctaatatcatttccaacatttcttcttctgtcagtgcatctgctcctggtgcttctggatgtgaggtcatagtgcaagctctactcgaagtcatcactgctcttgttcaaatcgttagttcttctagtgttggatatattaatccatctgctgtgaaccaaattactaatgttgttgctaatgccatggctcaagtaatgggc

SEQ ID NO: 25 - protein, 286 aa, Artificial Sequence
  Fusion protein
GPNSWWWWGRRPRPRPRPGPAALGSASGQGGYGGLGQGGYGQGAGSSAAAAAAAAAAAAGGQGGQGQGGYGQGSGGSAAAAAAAAAAAAAAAGRGQGGYGQGSGGNAAAAAAAAAAAAAAAGQGGQGGYGRQSQGAGSAAAAAAAAAAAAAAGSGQGGYGGQGQGGYGQSSASASAAASAASTVANSVSRLSSPSAVSRVSSAVSSLVSNGQVNMAALPNIISNISSSVSASAPGASGCEVIVQALLEVITALVQIVSSSSVGYINPSAVNQITNVVANAMAQVMG

SEQ ID NO: 26 - DNA, 858 bp, Artificial Sequence
  Fusion protein
ggtccgaattcatggtggtggtggggccgccgcccgcgcccgcgcccgcgcccgggcccggcggcgctgggatccgctagcggtcaaggaggatatggtggactaggtcaaggagggtatggacaaggtgcaggaagttctgcagccgctgccgccgccgcagcagccgccgcagcaggtggacaaggtggacaaggtcaaggaggatatggacaaggttcaggaggttctgcagccgccgccgccgccgcagcagcagcagcagctgcagcagctggacgaggtcaaggaggatatggccaaggttctggaggtaatgctgctgccgcagccgctgccgccgccgccgccgctgcagcagccggacagggaggtcaaggtggatatggtagacaaagccaaggtgctggttccgctgctgctgctgctgctgctgctgccgctgctgctgctgcaggatctggacaaggtggatacggtggacaaggtcaaggaggttatggtcagagtagtgcttctgcttcagctgctgcgtcagctgctagtactgtagctaattcggtgagtcgcctctcatcgccttccgcagtatctcgagtttcttcagcagtttctagcttggtttcaaatggtcaagtgaatatggcagcgttacctaatatcatttccaacatttcttcttctgtcagtgcatctgctcctggtgcttctggatgtgaggtcatagtgcaagctctactcgaagtcatcactgctcttgttcaaatcgttagttcttctagtgttggatatattaatccatctgctgtgaaccaaattactaatgttgttgctaatgccatggctcaagtaatgggc

SEQ ID NO: 27 - protein, 459 aa, Artificial Sequence
  Fusion protein
MGSSGHHHHHHMASTDYWQNWTDGGGIVNAVNGSGGNYSVNWSNTGNFVVGKGWTTGSPFRTINYNAGVWAPNGNGYLTLYGWTRSPLIEYYVVDSWGTYRPTGTYKGTVKSDGGTYDIYTTTRYNAPSIDGDRTTFTQYWSVRQSKRPTGSNATITFSNHVNAWKSHGMNLGSNWAYQVMATEGYQSSGSSNVTVWPNSGQGGYGGLGQGGYGQGAGSSAAAAAAAAAAAAGGQGGQGQGGYGQGSGGSAAAAAAAAAAAAAAAGRGQGGYGQGSGGNAAAAAAAAAAAAAAAGQGGQGGYGRQSQGAGSAAAAAAAAAAAAAAGSGQGGYGGQGQGGYGQSSASASAAASAASTVANSVSRLSSPSAVSRVSSAVSSLVSNGQVNMAALPNIISNISSSVSASAPGASGCEVIVQALLEVITALVQIVSSSSVGYINPSAVNQITNVVANAMAQVMG

SEQ ID NO: 28 - DNA, 1377 bp, Artificial Sequence
  Fusion protein
atgggcagcagcggccatcatcatcatcatcatatggctagcacagactactggcaaaattggactgatgggggcggtatagtaaacgctgtcaatgggtctggcgggaattacagtgttaattggtctaataccggaaattttgttgttggtaaaggttggactacaggttcgccatttaggacgataaactataatgccggagtttgggcgccgaatggcaatggatatttaactttatatggttggacgagatcacctctcatagaatattatgtagtggattcatggggtacttatagacctactggaacgtataaaggtactgtaaaaagtgatgggggtacgtatgacatatatacaactacacgttataacgcaccttccattgatggcgatcgcactacttttacgcagtactggagtgttcgccagtcgaagagaccaaccggaagcaacgctacaatcactttcagcaatcatgtgaacgcatggaagagccatggaatgaatctgggcagtaattgggcttaccaagtcatggcgacagaaggatatcaaagtagtggaagttctaacgtaacagtgtggccgaattcaggtcaaggtggatatggtggactaggtcaaggaggatatggacaaggtgcaggaagttctgcagccgctgccgccgccgcagcagccgccgcagcaggtggacaaggtggacaaggtcaaggaggatatggacaaggttcaggaggttctgcagccgccgccgccgccgcagcagcagcagcagctgcagcagctggacgaggtcaaggaggatatggtcaaggttctggaggtaatgctgctgccgcagccgctgccgccgccgccgccgctgcagcagccggacagggaggtcaaggtggatatggtagacaaagccaaggtgctggttccgctgctgctgctgctgctgctgctgccgctgctgctgctgcaggatctggacaaggtggatacggtggacaaggtcaaggaggttatggtcagagtagtgcttctgcttcagctgctgcgtcagctgctagtactgtagctaattcggtgagtcgcctctcatcgccttccgcagtatctcgagtttcttcagcagtttctagcttggtttcaaatggtcaagtgaatatggcagcgttacctaatatcatttccaacatttcttcttctgtcagtgcatctgctcctggtgcttctggatgtgaggtcatagtgcaagctctactcgaagtcatcactgctcttgttcaaatcgttagttcttctagtgttggatatattaatccatctgctgtgaaccaaattactaatgttgttgctaatgccatggctcaagtaatgggc

SEQ ID NO: 29 - protein, 433 aa, Artificial Sequence
  Fusion protein
MGSSGHHHHHHMDPSKDSKAQVSAAEAGITGTWYNQLGSTFIVTAGADGALTGTYESAVGNAESRYTLTGRYDSAPATDGSGTALGWRVAWKNNYRNAHSATTWSGQYVGGAEARINTQWTLTSGTTEANAWKSTLRGHDTFTKVKPSAASIDAAKKAGVNNGNPLDAVQQGNSGQGGYGGLGQGGYGQGAGSSAAAAAAAAAAAAGGQGGQGQGGYGQGSGGSAAAAAAAAAAAAAAAGRGQGGYGQGSGGNAAAAAAAAAAAAAAAGQGGQGGYGRQSQGAGSAAAAAAAAAAAAAAGSGQGGYGGQGQGGYGQSSASASAAASAASTVANSVSRLSSPSAVSRVSSAVSSLVSNGQVNMAALPNIISNISSSVSASAPGASGCEVIVQALLEVITALVQIVSSSSVGYINPSAVNQITNVVANAMAQVMG

SEQ ID NO: 30 - DNA, 1299 bp, Artificial Sequence
  Fusion protein
atgggcagcagcggccatcatcatcatcatcatatggatccgagcaaagatagcaaagcgcaggtgagcgcggcggaagcgggcattaccggcacctggtataaccagctgggcagcacctttattgtgaccgcgggcgcggatggcgcgctgaccggcacctatgaaagcgcggtgggcaacgcggaaagccgctataccctgaccggccgctatgatagcgcgccggcgaccgatggcagcggcaccgcgctgggctggcgcgtggcgtggaaaaacaactatcgcaacgcgcatagcgcgaccacctggagcggccagtatgtgggcggcgcggaagcgcgcattaacacccagtggaccctgaccagcggcaccaccgaagcgaacgcgtggaaaagcaccctgcgcggccatgatacctttaccaaagtgaaaccgagcgcggcgagcattgatgcggcgaaaaaagcgggcgtgaacaacggcaacccgctggatgcggtgcagcaggggaattcaggtcaaggtggatatggtggactaggtcaaggaggatatggacaaggtgcaggaagttctgcagccgctgccgccgccgcagcagccgccgcagcaggtggacaaggtggacaaggtcaaggaggatatggacaaggttcaggaggttctgcagccgccgccgccgccgcagcagcagcagcagctgcagcagctggacgaggtcaaggaggatatggtcaaggttctggaggtaatgctgctgccgcagccgctgccgccgccgccgccgctgcagcagccggacagggaggtcaaggtggatatggtagacaaagccaaggtgctggttccgctgctgctgctgctgctgctgctgccgctgctgctgctgcaggatctggacaaggtggatacggtggacaaggtcaaggaggttatggtcagagtagtgcttctgcttcagctgctgcgtcagctgctagtactgtagctaattcggtgagtcgcctctcatcgccttccgcagtatctcgagtttcttcagcagtttctagcttggtttcaaatggtcaagtgaatatggcagcgttacctaatatcatttccaacatttcttcttctgtcagtgcatctgctcctggtgcttctggatgtgaggtcatagtgcaagctctactcgaagtcatcactgctcttgttcaaatcgttagttcttctagtgttggatatattaatccatctgctgtgaaccaaattactaatgttgttgctaatgccatggctcaagtaatgggc

SEQ ID NO: 31 - protein, 18 aa, Euprosthenops australis
ASASAAASAASTVANSVS

SEQ ID NO: 32 - protein, 8 aa, Euprosthenops australis
ASAASAAA

SEQ ID NO: 33 - protein, 8 aa, Euprosthenops australis
GSAMGQGS

SEQ ID NO: 34 - protein, 5 aa, Euprosthenops australis
SASAG

SEQ ID NO: 35 - protein, 5 aa, Artificial Sequence
  cell-binding peptide
IKVAV

SEQ ID NO: 36 - protein, 5 aa, Artificial Sequence
  cell-binding peptide
YIGSR

SEQ ID NO: 37 - protein, 10 aa, Artificial Sequence
  cell-binding peptide
  misc_feature: X = any amino acid
  misc_feature (2)..(3): Xaa can be any naturally occurring amino acid
  misc_feature (7)..(9): Xaa can be any naturally occurring amino acid
CXXRGDXXXC

SEQ ID NO: 38 - protein, 100 aa, Euprosthenops sp
SRLSSPEASSRVSSAVSNLVSSGPTNSAALSSTISNVVSQIGASNPGLSGCDVLVQALLEVVSALIHILGSSSIGQVNYGSAGQATQLVGQSVYQALGEF

SEQ ID NO: 39 - protein, 98 aa, Euprosthenops australis; identical to SEQ ID NO: 3

SEQ ID NO: 40 - protein, 99 aa, Argiope trifasciata
SRLSSPGAASRVSSAVTSLVSSGGPTNSAALSNTISNVVSQISSSNPGLSGCDVLVQALLEIVSALVHILGSANIGQVNSSGVGRSASIVGQSINQAFS

SEQ ID NO: 41 - protein, 89 aa, Cyrtophora moluccensis
SHLSSPEASSRVSSAVSNLVSSGSTNSAALPNTISNVVSQISSSNPGLSGCDVLVQALLEVVSALIHILGSSSIGQVNYGSAGQATQIV

SEQ ID NO: 42 - protein, 98 aa, Latrodectus geometricus
SALAAPATSARISSHASTLLSNGPTNPASISNVISNAVSQISSSNPGASSCDVLVQALLELVTALLTIIGSSNVGNVNYDSSGQYAQVVSQSVQNAFV

SEQ ID NO: 43 - protein, 98 aa, Latrodectus hesperus
SALSAPATSARISSHASALLSSGPTNPASISNVISNAVSQISSSNPGASACDVLVQALLELVTALLTIIGSSNIGSVNYDSSGQYAQVVTQSVQNVFG

SEQ ID NO: 44 - protein, 93 aa, Macrothele holsti
SHLSSPEASSRVSSAVSNLVSGGSTNSAALPNTISNVVSQISSSNPGLSGCDVLVQALLEVVSALIHILGSSSIGQVDYGSAGQATQIVGQSA

SEQ ID NO: 45 - protein, 98 aa, Nephila clavipes
SRLSSPQASSRVSSAVSNLVASGPTNSAALSSTISNVVSQIGASNPGLSGCDVLIQALLEVVSALIQILGSSSIGQVNYGSAGQATQIVGQSVYQALG

SEQ ID NO: 46 - protein, 89 aa, Nephila pilipes
SRLSSPEASSRVSSAVSNLVSSGPTNSAALSNTISNVVSQISSSNPGLSGCDVLVQALLEVVSALIHILGSSSIGQVNYGSAGQATQIV

SEQ ID NO: 47 - protein, 87 aa, Nephila madagascariensis
SRLSSPQASSRVSSAVSNLVASGPTNSAALSSTISNAVSQIGASNPGLSGCDVLIQALLEVVSALIHILGSSSIGQVNYGSAGQATQ

SEQ ID NO: 48 - protein, 87 aa, Nephila senegalensis
SRLSSPEASSRVSSAVSNLVSSGPTNSAALSSTISNVVSQIGASNPGLSGCDVLIQALLEVVSALVHILGSSSIGQVNYGSAGQATQ

SEQ ID NO: 49 - protein, 89 aa, Octonoba varians
SRLSSPEASSRVSSAVSNLVSSGPTNSAALSNTISNVVSQISSSNPGLSGCDVLVQALLEVVSAPIHILGSSSIGQVNYGSAGQATQIV

SEQ ID NO: 50 - protein, 89 aa, Psechrus sinensis
SRLSSPEASSRVSSAVSNLVSSGPTNSAALPNTISNVVSQISSSNPGLSGCDVLVQALLEVVSALIHILGSSSIGQVNYGSAGQATQIV

SEQ ID NO: 51 - protein, 88 aa, Tetragnatha kauaiensis
SLLSSPASNARISSAVSALASGAASGPGYLSSVISNVVSQVSSNSGGLVGCDTLVQALLEAAAALVHVLASSSGGQVNLNTAGYTSQL

SEQ ID NO: 52 - protein, 88 aa, Tetragnatha versicolor
SRLSSPASNARISSAVSALASGGASSPGYLSSIISNVVSQVSSNNDGLSGCDTVVQALLEVAAALVHVLASSNIGQVNLNTAGYTSQL

SEQ ID NO: 53 - protein, 89 aa, Araneus bicentenarius
SRLSSSAASSRVSSAVSSLVSSGPTTPAALSNTISSAVSQISASNPGLSGCDVLVQALLEVVSALVHILGSSSVGQINYGASAQYAQMV

SEQ ID NO: 54 - protein, 97 aa, Argiope amoena
RLSSPQASSRVSSAVSTLVSSGPTNPASLSNAIGSVVSQVSASNPGLPSCDVLVQALLEIVSALVHILGSSSIGQINYSASSQYARLVGQSIAQALG

SEQ ID NO: 55 - protein, 82 aa, Argiope aurantia
SRLSSPQASSRVSSAVSTLVSSGPTNPAALSNAISSVVSQVSASNPGLSGCDVLVQALLELVSALVHILGSSSIGQINYAAS

SEQ ID NO: 56 - protein, 98 aa, Argiope trifasciata
SRLSSPQASSRVSSAVSTLVSSGPTNPASLSNAISSVVSQVSSSNPGLSGCDVLVQALLEIVSALVHILGSSSIGQINYAASSQYAQLVGQSLTQALG

SEQ ID NO: 57 - protein, 89 aa, Gasteracantha mammosa
SRLSSPQAGARVSSAVSALVASGPTSPAAVSSAISNVASQISASNPGLSGCDVLVQALLEIVSALVSILSSASIGQINYGASGQYAAMI

SEQ ID NO: 58 - protein, 90 aa, Latrodectus geometricus
SALSSPTTHARISSHASTLLSSGPTNSAAISNVISNAVSQVSASNPGSSSCDVLVQALLELITALISIVDSSNIGQVNYGSSGQYAQMVG

SEQ ID NO: 59 - protein, 98 aa, Latrodectus hesperus
SALSSPTTHARISSHASTLLSSGPTNAAALSNVISNAVSQVSASNPGSSSCDVLVQALLEIITALISILDSSSVGQVNYGSSGQYAQIVGQSMQQAMG

SEQ ID NO: 60 - protein, 97 aa, Nephila clavipes
SRLASPDSGARVASAVSNLVSSGPTSSAALSSVISNAVSQIGASNPGLSGCDVLIQALLEIVSACVTILSSSSIGQVNYGAASQFAQVVGQSVLSAF

SEQ ID NO: 61 - protein, 82 aa, Nephila madagascariensis
SRLASPDSGARVASAVSNLVSSGPTSSAALSSVISNAVSQIGASNPGLSGCDVLIQALLEIVSACVTILSSSSIGQVNYGAA

SEQ ID NO: 62 - protein, 82 aa, Nephila senegalensis
  misc_feature (35)..(35): Xaa can be any naturally occurring amino acid
  misc_feature (56)..(56): Xaa can be any naturally occurring amino acid
SRLASPDSGARVASAVSNLVSSGPTSSAALSSVIXNAVSQIGASNPGLSGCDVLIXALLEIVSACVTILSSSSIGQVNYGAA

SEQ ID NO: 63 - protein, 71 aa, Dolomedes tenebrosus
SRLSSPEAASRVSSAVSSLVSNGQVNVDALPSIISNLSSSISASATTASDCEVLVQVLLEVVSALVQIVCS

SEQ ID NO: 64 - protein, 97 aa, Dolomedes tenebrosus
SRLSSPQAASRVSSAVSSLVSNGQVNVAALPSIISSLSSSISASSTAASDCEVLVQVLLEIVSALVQIVSSANVGYINPEASGSLNAVGSALAAAMG

SEQ ID NO: 65 - protein, 93 aa, Araneus diadematus
NRLSSAGAASRVSSNVAAIASAGAAALPNVISNIYSGVLSSGVSSSEALIQALLEVISALIHVLGSASIGNVSSVGVNSALNAVQNAVGAYAG

SEQ ID NO: 66 - protein, 98 aa, Araneus diadematus
SRLSSPSAAARVSSAVSLVSNGGPTSPAALSSSISNVVSQISASNPGLSGCDILVQALLEIISALVHILGSANIGPVNSSSAGQSASIVGQSVYRALS

SEQ ID NO: 67 - protein, 98 aa, Araneus diadematus
SRLSSPAASSRVSSAVSSLVSSGPTKHAALSNTISSVVSQVSASNPGLSGCDVLVQALLEVVSALVSILGSSSIGQINYGASAQYTQMVGQSVAQALA

SEQ ID NO: 68 - protein, 94 aa, Araneus diadematus
SVYLRLQPRLEVSSAVSSLVSSGPTNGAAVSGALNSLVSQISASNPGLSGCDALVQALLELVSALVAILSSASIGQVNVSSVSQSTQMISQALS

SEQ ID NO: 69 - protein, 93 aa, Araneus ventricosus
NRLSSAEAASRVSSNIAAIASGGASALPSVISNIYSGVVASGVSSNEALIQALLELLSALVHVLSSASIGNVSSVGVDSTLNVVQDSVGQYVG

SEQ ID NO: 70 - protein, 272 aa, Artificial Sequence
  Fusion protein
GPNSCTGRGDSPACGSASGQGGYGGLGQGGYGQGAGSSAAAAAAAAAAAAGGQGGQGQGGYGQGSGGSAAAAAAAAAAAAAAAGRGQGGYGQGSGGNAAAAAAAAAAAAAAAGQGGQGGYGRQSQGAGSAAAAAAAAAAAAAAGSGQGGYGGQGQGGYGQSSASASAAASAAGSYAGAVNRLSSAEAASRVSSNIAAIASGGASALPSVISNIYSGVVASGVSSNEALIQALLELLSALVHVLSSASIGNVSSVGVDSTLNVVQDSVGQYVG

SEQ ID NO: 71 - protein, 151 aa, Euprosthenops australis
GSGNSGIQGQGGYGGLGQGGYGQGAGSSAAAAAAAAAAAAGGQGGQGQGGYGQGSGGSAAAAAAAAAAAAAAAGRGQGGYGQGSGGNAAAAAAAAAAAAAAAGQGGQGGYGRQSQGAGSAAAAAAAAAAAAAAGSGQGGYGGQGQGGYGQS

SEQ ID NO: 72 - protein, 270 aa, Artificial Sequence
  Fusion protein
GPNSRGDAGAASGQGGYGGLGQGGYGQGAGSSAAAAAAAAAAAAGQGGQGQGGYGQGSGGSAAAAAAAAAAAAAAAGRGQGGYGQGSGGNAAAAAAAAAAAAAAAGQGGQGGYGRQSQGAGSAAAAAAAAAAAAAAGSGQGGYGGQGQGGYGQSSASASAAASAASTVANSVSRLSSPSAVSRVSSAVSSLVSNGQVNMAALPNIISNISSSVSASAPGASGCEVIVQALLEVITALVQIVSSSSVGYINPSAVNQITNVVANAMAQVMG